European Patent Application EP 4 700 121 A1, published February 25, 2026. Title: DON 분해 활성을 갖는 신규 폴리펩티드. Applicant: 씨제이제일제당 주식회사. The sequence listing filed with the application follows.

SEQUENCE LISTING (31 sequences)

SEQ ID NO: 1 - protein, 181 aa, synthetic construct
MASSDLKESAANNPGLHTTPDEATKDYIMQQTMYRIKDPKVSLDFYSRVLGMSLLKRVDVPELKFTLYFMGYEDVSKAPSDPYGRTVWTFGRAATIELTHNWGTESDPEFKGYHTGNSEPRGFGHIGITVDDVNKACERFERLGVEFVKKPSDGFAFIKDPDGYWIEIFDLKTIGDIQRVL

SEQ ID NO: 2 - DNA, 546 bp, synthetic construct
  source 1..546: mol_type = other DNA
atggcgagttcagatcttaaagaaagcgccgccaataaccccggattacacacgactccggatgaggcaaccaaggattacattatgcaacagaccatgtatcggataaaggaccctaaggtaagtcttgacttttattcgcgggtccttggcatgagtctgcttaagcgggtcgacgttcccgagctgaaatttacactttattttatggggtacgaggacgtgtccaaagccccgtctgatccttacggacgcacagtctggacttttggtcgtgctgcaacgattgaactgacgcacaactggggcactgagagtgacccagagttcaaaggttatcacacgggaaatagtgaaccacggggattcggtcacatagggatcaccgtggatgatgtcaataaggcgtgcgaaagattcgagagattaggggtcgaatttgtgaaaaaaccgtctgatggctttgctttcattaaagatcctgatggatattggattgagattttcgatctgaagaccataggcgacattcagcgcgtattataa

SEQ ID NO: 3 - protein, 182 aa, synthetic construct
MASSGPKESAANNPGLQTPPDEATKGYFMQQTMFRIKDPKVSLDFYSRVLGMSLLKRIDVPDMKFTLYFMGYEDVSSAPSDPIERTAWTFGRPATIELTHKWGTESDPEFKGYHNGNSEPRGFGHIGITVDDTYKACERFERLGVEFVKKPDDGYAFIKDPDGYWIEIFDLKNIRNVVNGVA

SEQ ID NO: 4 - DNA, 546 bp, synthetic construct
  source 1..546: mol_type = other DNA
atggcatcgtccgggccgaaagagtcggctgccaataatcctggcttgcaaactccacctgacgaggccactaagggttattttatgcaacagacaatgtttcgcattaaagaccctaaagtgtctttggacttctattcgcgcgtgcttggtatgagccttttgaaaagaattgacgtcccggatatgaagttcacgttatattttatgggatatgaagatgtaagtagtgcgccaagtgatccaatagagcggaccgcctggacatttggcagaccagcgacaatcgaattgacccataagtggggtaccgagagcgacccggagtttaaaggttaccataatggcaattctgaaccacggggtttcgggcacataggcatcacggtcgatgacacttacaaggcgtgtgagagattcgaacgtcttggggtagaatttgtgaaaaagccggatgacggctatgcgtttattaaagaccccgatggctactggatagagatatttgacttgaagaatatacgcaatgtggtaaatggagtcgct

SEQ ID NO: 5 - protein, 181 aa, synthetic construct
MASSDLKESAANNPGLHTTPDEATKDYIMQQTMYRIKDPKVSLDFYSRVLGMSLLKRVDVPELKMTLYFMGYEDVSKAPSDPYGRTVWTFGRAATIELTHNWGTESDPEFKGYHTGNSEPRGFGHIGITVDDVNKACERFERLGVEFVKKPSDGFAFIKDPDGYWIEIFDLKTIGDIQRVL

SEQ ID NO: 6 - DNA, 546 bp, synthetic construct
  source 1..546: mol_type = other DNA
atggcgagttcagatcttaaagaaagcgccgccaataaccccggattacacacgactccggatgaggcaaccaaggattacattatgcaacagaccatgtatcggataaaggaccctaaggtaagtcttgacttttattcgcgggtccttggcatgagtctgcttaagcgggtcgacgttcccgagctgaaaatgacactttattttatggggtacgaggacgtgtccaaagccccgtctgatccttacggacgcacagtctggacttttggtcgtgctgcaacgattgaactgacgcacaactggggcactgagagtgacccagagttcaaaggttatcacacgggaaatagtgaaccacggggattcggtcacatagggatcaccgtggatgatgtcaataaggcgtgcgaaagattcgagagattaggggtcgaatttgtgaaaaaaccgtctgatggctttgctttcattaaagatcctgatggatattggattgagattttcgatctgaagaccataggcgacattcagcgcgtattataa

SEQ ID NO: 7 - protein, 181 aa, synthetic construct
MASSDLKESAANNPGLHTTPDEATKDYIMQQTMYRIKDPKVSLDFYSRVLGMSLLKRVDVPELKFTLYFMGYEDVSKAPSDPYGRTVWTFGRAATIELTHNWGTESDPEFKGYHTGNSEPIGFGHIGITVDDVNKACERFERLGVEFVKKPSDGFAFIKDPDGYWIEIFDLKTIGDIQRVL

SEQ ID NO: 8 - DNA, 546 bp, synthetic construct
  source 1..546: mol_type = other DNA
atggcgagttcagatcttaaagaaagcgccgccaataaccccggattacacacgactccggatgaggcaaccaaggattacattatgcaacagaccatgtatcggataaaggaccctaaggtaagtcttgacttttattcgcgggtccttggcatgagtctgcttaagcgggtcgacgttcccgagctgaaatttacactttattttatggggtacgaggacgtgtccaaagccccgtctgatccttacggacgcacagtctggacttttggtcgtgctgcaacgattgaactgacgcacaactggggcactgagagtgacccagagttcaaaggttatcacacgggaaatagtgaaccaattggattcggtcacatagggatcaccgtggatgatgtcaataaggcgtgcgaaagattcgagagattaggggtcgaatttgtgaaaaaaccgtctgatggctttgctttcattaaagatcctgatggatattggattgagattttcgatctgaagaccataggcgacattcagcgcgtattataa

SEQ ID NO: 9 - protein, 182 aa, synthetic construct
MASSGPKESAANNPGLQTPPDEATKGYFMQQTMFRIKDPKVSLDFYSRVLGMSLLKRIDVPDMKMTLYFMGYEDVSSAPSDPIERTAWTFGRPATIELTHKWGTESDPEFKGYHNGNSEPRGFGHIGITVDDTYKACERFERLGVEFVKKPDDGYAFIKDPDGYWIEIFDLKNIRNVVNGVA

SEQ ID NO: 10 - DNA, 546 bp, synthetic construct
  source 1..546: mol_type = other DNA
atggcatcgtccgggccgaaagagtcggctgccaataatcctggcttgcaaactccacctgacgaggccactaagggttattttatgcaacagacaatgtttcgcattaaagaccctaaagtgtctttggacttctattcgcgcgtgcttggtatgagccttttgaaaagaattgacgtcccggatatgaagatgacgttatattttatgggatatgaagatgtaagtagtgcgccaagtgatccaatagagcggaccgcctggacatttggcagaccagcgacaatcgaattgacccataagtggggtaccgagagcgacccggagtttaaaggttaccataatggcaattctgaaccacggggtttcgggcacataggcatcacggtcgatgacacttacaaggcgtgtgagagattcgaacgtcttggggtagaatttgtgaaaaagccggatgacggctatgcgtttattaaagaccccgatggctactggatagagatatttgacttgaagaatatacgcaatgtggtaaatggagtcgct

SEQ ID NO: 11 - protein, 182 aa, synthetic construct
MASSGPKESAANNPGLQTPPDEATKGYFMQQTMFRIKDPKVSLDFYSRVLGMSLLKRIDVPDMKFTLYFMGYEDVSSAPSDPIERTAWTFGRPATIELTHKWGTESDPEFKGYHNGNSEPIGFGHIGITVDDTYKACERFERLGVEFVKKPDDGYAFIKDPDGYWIEIFDLKNIRNVVNGVA

SEQ ID NO: 12 - DNA, 546 bp, synthetic construct
  source 1..546: mol_type = other DNA
atggcatcgtccgggccgaaagagtcggctgccaataatcctggcttgcaaactccacctgacgaggccactaagggttattttatgcaacagacaatgtttcgcattaaagaccctaaagtgtctttggacttctattcgcgcgtgcttggtatgagccttttgaaaagaattgacgtcccggatatgaagttcacgttatattttatgggatatgaagatgtaagtagtgcgccaagtgatccaatagagcggaccgcctggacatttggcagaccagcgacaatcgaattgacccataagtggggtaccgagagcgacccggagtttaaaggttaccataatggcaattctgaaccaattggtttcgggcacataggcatcacggtcgatgacacttacaaggcgtgtgagagattcgaacgtcttggggtagaatttgtgaaaaagccggatgacggctatgcgtttattaaagaccccgatggctactggatagagatatttgacttgaagaatatacgcaatgtggtaaatggagtcgct

SEQ ID NO: 13 - DNA, 44 bp, synthetic construct
  source 1..44: mol_type = other DNA
acgttcccgagctgaaaatgacactttattttatggggtacgag

SEQ ID NO: 14 - DNA, 43 bp, synthetic construct
  source 1..43: mol_type = other DNA
cattttcagctcgggaacgtcgacccgcttaagcagactcatg

SEQ ID NO: 15 - DNA, 45 bp, synthetic construct
  source 1..45: mol_type = other DNA
attggattcggtcacatagggatcaccgtggatgatgtcaataag

SEQ ID NO: 16 - DNA, 42 bp, synthetic construct
  source 1..42: mol_type = other DNA
ccctatgtgaccgaatccaattggttcactatttcccgtgtg

SEQ ID NO: 17 - DNA, 41 bp, synthetic construct
  source 1..41: mol_type = other DNA
cccggatatgaagatgacgttatattttatgggatatgaag

SEQ ID NO: 18 - DNA, 40 bp, synthetic construct
  source 1..40: mol_type = other DNA
acgtcatcttcatatccgggacgtcaattcttttcaaaag

SEQ ID NO: 19 - DNA, 42 bp, synthetic construct
  source 1..42: mol_type = other DNA
atcggtttcgggcacataggcatcacggtcgatgacacttac

SEQ ID NO: 20 - DNA, 42 bp, synthetic construct
  source 1..42: mol_type = other DNA
cctatgtgcccgaaaccgattggttcagaattgccattatgg

SEQ ID NO: 21 - protein, 185 aa, Punica granatum SPG
MASEPKESPANNPGLHSTADEATKGYFMQQTMFRIKDPKVSLDFYSRVLGMSLLKRLDFPEMKFSLYFLGYEDTSSAPSNAVDRTVWTFGQKATIELTHNWGTESDPEFKGYHNGNSDPRGFGHIGITVDDTYKACERFERLGVEFVKKPDDGKMKGIAFIKDPDGYWIEIFDLKTIGKVTEAAA

SEQ ID NO: 22 - protein, 185 aa, synthetic construct
MASESKESPANNPGLCSTPDEATKGYFMQQTMFRIKDPKVSLDFYSRVLGMSLLKRLDFPEMKFSLYFMGYEDTASAPSDPTERTAWTFGQKATLELTHNWGTESDPEFKGYHNGNSEPRGFGHIGITVDDVYKACERFERLGVEFVKKPDDGKMKGIAFIKDPDGYWIEIFDLKNIKSVTSAAS

SEQ ID NO: 23 - DNA, 555 bp, synthetic construct
  source 1..555: mol_type = other DNA
atggcaagcgagtcgaaagagagcccggcgaacaaccctggcttatgttcgacgccagacgaggcaaccaaaggttattttatgcagcaaaccatgttccgtatcaaagaccctaaggtgagtttggacttttacagtcgtgttcttggaatgagcctgttgaaaagactggactttccagaaatgaagtttagtctttattttatgggttatgaagatacagcatccgcacccagcgacccgaccgaacggactgcttggacttttgggcagaaggctaccttggagttgactcataattgggggacagagagcgacccggagttcaaaggatatcacaacggaaatagcgaaccaagaggctttggccacataggaatcacggtggacgacgtctacaaggcatgtgagcggttcgagcggttaggggtcgaatttgtaaaaaagccagacgacgggaagatgaagggaatcgcgtttattaaagatccggatggttattggatagaaatcttcgaccttaaaaatatcaagagtgtaacgtcagccgcgagc

SEQ ID NO: 24 - protein, 185 aa, synthetic construct
MASESKESPANNPGLCSTPDEATKGYFMQQTMFRIKDPKVSLDFYSRVLGMSLLKRLDFPEMKMSLYFMGYEDTASAPSDPTERTAWTFGQKATLELTHNWGTESDPEFKGYHNGNSEPRGFGHIGITVDDVYKACERFERLGVEFVKKPDDGKMKGIAFIKDPDGYWIEIFDLKNIKSVTSAAS

SEQ ID NO: 25 - DNA, 555 bp, synthetic construct
  source 1..555: mol_type = other DNA
atggcaagcgagtcgaaagagagcccggcgaacaaccctggcttatgttcgacgccagacgaggcaaccaaaggttattttatgcagcaaaccatgttccgtatcaaagaccctaaggtgagtttggacttttacagtcgtgttcttggaatgagcctgttgaaaagactggactttccagaaatgaagatgagtctttattttatgggttatgaagatacagcatccgcacccagcgacccgaccgaacggactgcttggacttttgggcagaaggctaccttggagttgactcataattgggggacagagagcgacccggagttcaaaggatatcacaacggaaatagcgaaccaagaggctttggccacataggaatcacggtggacgacgtctacaaggcatgtgagcggttcgagcggttaggggtcgaatttgtaaaaaagccagacgacgggaagatgaagggaatcgcgtttattaaagatccggatggttattggatagaaatcttcgaccttaaaaatatcaagagtgtaacgtcagccgcgagc

SEQ ID NO: 26 - protein, 185 aa, synthetic construct
MASESKESPANNPGLCSTPDEATKGYFMQQTMFRIKDPKVSLDFYSRVLGMSLLKRLDFPEMKFSLYFMGYEDTASAPSDPTERTAWTFGQKATLELTHNWGTESDPEFKGYHNGNSEPIGFGHIGITVDDVYKACERFERLGVEFVKKPDDGKMKGIAFIKDPDGYWIEIFDLKNIKSVTSAAS

SEQ ID NO: 27 - DNA, 555 bp, synthetic construct
  source 1..555: mol_type = other DNA
atggcaagcgagtcgaaagagagcccggcgaacaaccctggcttatgttcgacgccagacgaggcaaccaaaggttattttatgcagcaaaccatgttccgtatcaaagaccctaaggtgagtttggacttttacagtcgtgttcttggaatgagcctgttgaaaagactggactttccagaaatgaagtttagtctttattttatgggttatgaagatacagcatccgcacccagcgacccgaccgaacggactgcttggacttttgggcagaaggctaccttggagttgactcataattgggggacagagagcgacccggagttcaaaggatatcacaacggaaatagcgaaccaattggctttggccacataggaatcacggtggacgacgtctacaaggcatgtgagcggttcgagcggttaggggtcgaatttgtaaaaaagccagacgacgggaagatgaagggaatcgcgtttattaaagatccggatggttattggatagaaatcttcgaccttaaaaatatcaagagtgtaacgtcagccgcgagc

SEQ ID NO: 28 - DNA, 49 bp, synthetic construct
  source 1..49: mol_type = other DNA
actttccagaaatgaagatgagtctttattttatgggttatgaagatac

SEQ ID NO: 29 - DNA, 44 bp, synthetic construct
  source 1..44: mol_type = other DNA
catcttcatttctggaaagtccagtcttttcaacaggctcattc

SEQ ID NO: 30 - DNA, 44 bp, synthetic construct
  source 1..44: mol_type = other DNA
acggaaatagcgaaccaattggctttggccacataggaatcacg

SEQ ID NO: 31 - DNA, 47 bp, synthetic construct
  source 1..47: mol_type = other DNA
aattggttcgctatttccgttgtgatatcctttgaactccgggtcgc